European Patent Application EP 4 159 243 A1, published April 5, 2023. Title: RNA-Guided Transcriptional Regulation. Applicant: President and Fellows of Harvard College. Application PCT/US14/040868. The sequence listing filed with the application follows.

SEQUENCE LISTING (184 sequences)

SEQ ID NO: 1 - protein, 1368 aa, Streptococcus pyogenes [sequence omitted]

SEQ ID NO: 2 - DNA, 4332 bp, Artificial
  VP64-activator construct
gccaccatggacaagaagtactccattgggctcgctatcggcacaaacagcgtcggctgggccgtcattacggacgagtacaaggtgccgagcaaaaaattcaaagttctgggcaataccgatcgccacagcataaagaagaacctcattggcgccctcctgttcgactccggggagacggccgaagccacgcggctcaaaagaacagcacggcgcagatatacccgcagaaagaatcggatctgctacctgcaggagatctttagtaatgagatggctaaggtggatgactctttcttccataggctggaggagtcctttttggtggaggaggataaaaagcacgagcgccacccaatctttggcaatatcgtggacgaggtggcgtaccatgaaaagtacccaaccatatatcatctgaggaagaagcttgtagacagtactgataaggctgacttgcggttgatctatctcgcgctggcgcatatgatcaaatttcggggacacttcctcatcgagggggacctgaacccagacaacagcgatgtcgacaaactctttatccaactggttcagacttacaatcagcttttcgaagagaacccgatcaacgcatccggagttgacgccaaagcaatcctgagcgctaggctgtccaaatcccggcggctcgaaaacctcatcgcacagctccctggggagaagaagaacggcctgtttggtaatcttatcgccctgtcactcgggctgacccccaactttaaatctaacttcgacctggccgaagatgccaagcttcaactgagcaaagacacctacgatgatgatctcgacaatctgctggcccagatcggcgaccagtacgcagacctttttttggcggcaaagaacctgtcagacgccattctgctgagtgatattctgcgagtgaacacggagatcaccaaagctccgctgagcgctagtatgatcaagcgctatgatgagcaccaccaagacttgactttgctgaaggcccttgtcagacagcaactgcctgagaagtacaaggaaattttcttcgatcagtctaaaaatggctacgccggatacattgacggcggagcaagccaggaggaattttacaaatttattaagcccatcttggaaaaaatggacggcaccgaggagctgctggtaaagcttaacagagaagatctgttgcgcaaacagcgcactttcgacaatggaagcatcccccaccagattcacctgggcgaactgcacgctatcctcaggcggcaagaggatttctacccctttttgaaagataacagggaaaagattgagaaaatcctcacatttcggataccctactatgtaggccccctcgcccggggaaattccagattcgcgtggatgactcgcaaatcagaagagaccatcactccctggaacttcgaggaagtcgtggataagggggcctctgcccagtccttcatcgaaaggatgactaactttgataaaaatctgcctaacgaaaaggtgcttcctaaacactctctgctgtacgagtacttcacagtttataacgagctcaccaaggtcaaatacgtcacagaagggatgagaaagccagcattcctgtctggagagcagaagaaagctatcgtggacctcctcttcaagacgaaccggaaagttaccgtgaaacagctcaaagaagactatttcaaaaagattgaatgtttcgactctgttgaaatcagcggagtggaggatcgcttcaacgcatccctgggaacgtatcacgatctcctgaaaatcattaaagacaaggacttcctggacaatgaggagaacgaggacattcttgaggacattgtcctcacccttacgttgtttgaagatagggagatgattgaagaacgcttgaaaacttacgctcatctcttcgacgacaaagtcatgaaacagctcaagaggcgccgatatacaggatgggggcggctgtcaagaaaactgatcaatgggatccgagacaagcagagtggaaagacaatcctggattttcttaagtccgatggatttgccaaccggaacttcatgcagttgatccatgatgactctctcacctttaaggaggacatccagaaagcacaagtttctggccagggggacagtcttcacgagcacatcgctaatcttgcaggtagcccagctatcaaaaagggaatactgcagaccgttaaggtcgtggatgaactcgtcaaagtaatgggaaggcataagcccgagaatatcgttatcgagatggcccgagagaaccaaactacccagaagggacagaagaacagtagggaaaggatgaagaggattgaagagggtataaaagaactggggtcccaaatccttaaggaacacccagttgaaaacacccagcttcagaatgagaagctctacctgtactacctgcagaacggcagggacatgtacgtggatcaggaactggacatcaatcggctctccgactacgacgtggctgctatcgtgccccagtcttttctcaaagatgattctattgataataaagtgttgacaagatccgataaagctagagggaagagtgataacgtcccctcagaagaagttgtcaagaaaatgaaaaattattggcggcagctgctgaacgccaaactgatcacacaacggaagttcgataatctgactaaggctgaacgaggtggcctgtctgagttggataaagccggcttcatcaaaaggcagcttgttgagacacgccagatcaccaagcacgtggcccaaattctcgattcacgcatgaacaccaagtacgatgaaaatgacaaactgattcgagaggtgaaagttattactctgaagtctaagctggtctcagatttcagaaaggactttcagttttataaggtgagagagatcaacaattaccaccatgcgcatgatgcctacctgaatgcagtggtaggcactgcacttatcaaaaaatatcccaagcttgaatctgaatttgtttacggagactataaagtgtacgatgttaggaaaatgatcgcaaagtctgagcaggaaataggcaaggccaccgctaagtacttcttttacagcaatattatgaattttttcaagaccgagattacactggccaatggagagattcggaagcgaccacttatcgaaacaaacggagaaacaggagaaatcgtgtgggacaagggtagggatttcgcgacagtccggaaggtcctgtccatgccgcaggtgaacatcgttaaaaagaccgaagtacagaccggaggcttctccaaggaaagtatcctcccgaaaaggaacagcgacaagctgatcgcacgcaaaaaagattgggaccccaagaaatacggcggattcgattctcctacagtcgcttacagtgtactggttgtggccaaagtggagaaagggaagtctaaaaaactcaaaagcgtcaaggaactgctgggcatcacaatcatggagcgatcaagcttcgaaaaaaaccccatcgactttctcgaggcgaaaggatataaagaggtcaaaaaagacctcatcattaagcttcccaagtactctctctttgagcttgaaaacggccggaaacgaatgctcgctagtgcgggcgagctgcagaaaggtaacgagctggcactgccctctaaatacgttaatttcttgtatctggccagccactatgaaaagctcaaagggtctcccgaagataatgagcagaagcagctgttcgtggaacaacacaaacactaccttgatgagatcatcgagcaaataagcgaattctccaaaagagtgatcctcgccgacgctaacctcgataaggtgctttctgcttacaataagcacagggataagcccatcagggagcaggcagaaaacattatccacttgtttactctgaccaacttgggcgcgcctgcagccttcaagtacttcgacaccaccatagacagaaagcggtacacctctacaaaggaggtcctggacgccacactgattcatcagtcaattacggggctctatgaaacaagaatcgacctctctcagctcggtggagacagcagggctgaccccaagaagaagaggaaggtggaggccagcggttccggacgggctgacgcattggacgattttgatctggatatgctgggaagtgacgccctcgatgattttgaccttgacatgcttggttcggatgcccttgatgactttgacctcgacatgctcggcagtgacgcccttgatgatttcgacctggacatgctgattaactctagatga

SEQ ID NO: 3 - DNA, 4365 bp, Artificial
  VP64-activator construct
gccaccatgcccaagaagaagaggaaggtgggaagggggatggacaagaagtactccattgggctcgctatcggcacaaacagcgtcggctgggccgtcattacggacgagtacaaggtgccgagcaaaaaattcaaagttctgggcaataccgatcgccacagcataaagaagaacctcattggcgccctcctgttcgactccggggagacggccgaagccacgcggctcaaaagaacagcacggcgcagatatacccgcagaaagaatcggatctgctacctgcaggagatctttagtaatgagatggctaaggtggatgactctttcttccataggctggaggagtcctttttggtggaggaggataaaaagcacgagcgccacccaatctttggcaatatcgtggacgaggtggcgtaccatgaaaagtacccaaccatatatcatctgaggaagaagcttgtagacagtactgataaggctgacttgcggttgatctatctcgcgctggcgcatatgatcaaatttcggggacacttcctcatcgagggggacctgaacccagacaacagcgatgtcgacaaactctttatccaactggttcagacttacaatcagcttttcgaagagaacccgatcaacgcatccggagttgacgccaaagcaatcctgagcgctaggctgtccaaatcccggcggctcgaaaacctcatcgcacagctccctggggagaagaagaacggcctgtttggtaatcttatcgccctgtcactcgggctgacccccaactttaaatctaacttcgacctggccgaagatgccaagcttcaactgagcaaagacacctacgatgatgatctcgacaatctgctggcccagatcggcgaccagtacgcagacctttttttggcggcaaagaacctgtcagacgccattctgctgagtgatattctgcgagtgaacacggagatcaccaaagctccgctgagcgctagtatgatcaagcgctatgatgagcaccaccaagacttgactttgctgaaggcccttgtcagacagcaactgcctgagaagtacaaggaaattttcttcgatcagtctaaaaatggctacgccggatacattgacggcggagcaagccaggaggaattttacaaatttattaagcccatcttggaaaaaatggacggcaccgaggagctgctggtaaagcttaacagagaagatctgttgcgcaaacagcgcactttcgacaatggaagcatcccccaccagattcacctgggcgaactgcacgctatcctcaggcggcaagaggatttctacccctttttgaaagataacagggaaaagattgagaaaatcctcacatttcggataccctactatgtaggccccctcgcccggggaaattccagattcgcgtggatgactcgcaaatcagaagagaccatcactccctggaacttcgaggaagtcgtggataagggggcctctgcccagtccttcatcgaaaggatgactaactttgataaaaatctgcctaacgaaaaggtgcttcctaaacactctctgctgtacgagtacttcacagtttataacgagctcaccaaggtcaaatacgtcacagaagggatgagaaagccagcattcctgtctggagagcagaagaaagctatcgtggacctcctcttcaagacgaaccggaaagttaccgtgaaacagctcaaagaagactatttcaaaaagattgaatgtttcgactctgttgaaatcagcggagtggaggatcgcttcaacgcatccctgggaacgtatcacgatctcctgaaaatcattaaagacaaggacttcctggacaatgaggagaacgaggacattcttgaggacattgtcctcacccttacgttgtttgaagatagggagatgattgaagaacgcttgaaaacttacgctcatctcttcgacgacaaagtcatgaaacagctcaagaggcgccgatatacaggatgggggcggctgtcaagaaaactgatcaatgggatccgagacaagcagagtggaaagacaatcctggattttcttaagtccgatggatttgccaaccggaacttcatgcagttgatccatgatgactctctcacctttaaggaggacatccagaaagcacaagtttctggccagggggacagtcttcacgagcacatcgctaatcttgcaggtagcccagctatcaaaaagggaatactgcagaccgttaaggtcgtggatgaactcgtcaaagtaatgggaaggcataagcccgagaatatcgttatcgagatggcccgagagaaccaaactacccagaagggacagaagaacagtagggaaaggatgaagaggattgaagagggtataaaagaactggggtcccaaatccttaaggaacacccagttgaaaacacccagcttcagaatgagaagctctacctgtactacctgcagaacggcagggacatgtacgtggatcaggaactggacatcaatcggctctccgactacgacgtggctgctatcgtgccccagtcttttctcaaagatgattctattgataataaagtgttgacaagatccgataaagctagagggaagagtgataacgtcccctcagaagaagttgtcaagaaaatgaaaaattattggcggcagctgctgaacgccaaactgatcacacaacggaagttcgataatctgactaaggctgaacgaggtggcctgtctgagttggataaagccggcttcatcaaaaggcagcttgttgagacacgccagatcaccaagcacgtggcccaaattctcgattcacgcatgaacaccaagtacgatgaaaatgacaaactgattcgagaggtgaaagttattactctgaagtctaagctggtctcagatttcagaaaggactttcagttttataaggtgagagagatcaacaattaccaccatgcgcatgatgcctacctgaatgcagtggtaggcactgcacttatcaaaaaatatcccaagcttgaatctgaatttgtttacggagactataaagtgtacgatgttaggaaaatgatcgcaaagtctgagcaggaaataggcaaggccaccgctaagtacttcttttacagcaatattatgaattttttcaagaccgagattacactggccaatggagagattcggaagcgaccacttatcgaaacaaacggagaaacaggagaaatcgtgtgggacaagggtagggatttcgcgacagtccggaaggtcctgtccatgccgcaggtgaacatcgttaaaaagaccgaagtacagaccggaggcttctccaaggaaagtatcctcccgaaaaggaacagcgacaagctgatcgcacgcaaaaaagattgggaccccaagaaatacggcggattcgattctcctacagtcgcttacagtgtactggttgtggccaaagtggagaaagggaagtctaaaaaactcaaaagcgtcaaggaactgctgggcatcacaatcatggagcgatcaagcttcgaaaaaaaccccatcgactttctcgaggcgaaaggatataaagaggtcaaaaaagacctcatcattaagcttcccaagtactctctctttgagcttgaaaacggccggaaacgaatgctcgctagtgcgggcgagctgcagaaaggtaacgagctggcactgccctctaaatacgttaatttcttgtatctggccagccactatgaaaagctcaaagggtctcccgaagataatgagcagaagcagctgttcgtggaacaacacaaacactaccttgatgagatcatcgagcaaataagcgaattctccaaaagagtgatcctcgccgacgctaacctcgataaggtgctttctgcttacaataagcacagggataagcccatcagggagcaggcagaaaacattatccacttgtttactctgaccaacttgggcgcgcctgcagccttcaagtacttcgacaccaccatagacagaaagcggtacacctctacaaaggaggtcctggacgccacactgattcatcagtcaattacggggctctatgaaacaagaatcgacctctctcagctcggtggagacagcagggctgaccccaagaagaagaggaaggtggaggccagcggttccggacgggctgacgcattggacgattttgatctggatatgctgggaagtgacgccctcgatgattttgaccttgacatgcttggttcggatgcccttgatgactttgacctcgacatgctcggcagtgacgcccttgatgatttcgacctggacatgctgattaactctagatga

SEQ ID NO: 4 - DNA, 4425 bp, Artificial
  VP64-activator construct
gccaccatggacaagaagtactccattgggctcgctatcggcacaaacagcgtcggctgggccgtcattacggacgagtacaaggtgccgagcaaaaaattcaaagttctgggcaataccgatcgccacagcataaagaagaacctcattggcgccctcctgttcgactccggggagacggccgaagccacgcggctcaaaagaacagcacggcgcagatatacccgcagaaagaatcggatctgctacctgcaggagatctttagtaatgagatggctaaggtggatgactctttcttccataggctggaggagtcctttttggtggaggaggataaaaagcacgagcgccacccaatctttggcaatatcgtggacgaggtggcgtaccatgaaaagtacccaaccatatatcatctgaggaagaagcttgtagacagtactgataaggctgacttgcggttgatctatctcgcgctggcgcatatgatcaaatttcggggacacttcctcatcgagggggacctgaacccagacaacagcgatgtcgacaaactctttatccaactggttcagacttacaatcagcttttcgaagagaacccgatcaacgcatccggagttgacgccaaagcaatcctgagcgctaggctgtccaaatcccggcggctcgaaaacctcatcgcacagctccctggggagaagaagaacggcctgtttggtaatcttatcgccctgtcactcgggctgacccccaactttaaatctaacttcgacctggccgaagatgccaagcttcaactgagcaaagacacctacgatgatgatctcgacaatctgctggcccagatcggcgaccagtacgcagacctttttttggcggcaaagaacctgtcagacgccattctgctgagtgatattctgcgagtgaacacggagatcaccaaagctccgctgagcgctagtatgatcaagcgctatgatgagcaccaccaagacttgactttgctgaaggcccttgtcagacagcaactgcctgagaagtacaaggaaattttcttcgatcagtctaaaaatggctacgccggatacattgacggcggagcaagccaggaggaattttacaaatttattaagcccatcttggaaaaaatggacggcaccgaggagctgctggtaaagcttaacagagaagatctgttgcgcaaacagcgcactttcgacaatggaagcatcccccaccagattcacctgggcgaactgcacgctatcctcaggcggcaagaggatttctacccctttttgaaagataacagggaaaagattgagaaaatcctcacatttcggataccctactatgtaggccccctcgcccggggaaattccagattcgcgtggatgactcgcaaatcagaagagaccatcactccctggaacttcgaggaagtcgtggataagggggcctctgcccagtccttcatcgaaaggatgactaactttgataaaaatctgcctaacgaaaaggtgcttcctaaacactctctgctgtacgagtacttcacagtttataacgagctcaccaaggtcaaatacgtcacagaagggatgagaaagccagcattcctgtctggagagcagaagaaagctatcgtggacctcctcttcaagacgaaccggaaagttaccgtgaaacagctcaaagaagactatttcaaaaagattgaatgtttcgactctgttgaaatcagcggagtggaggatcgcttcaacgcatccctgggaacgtatcacgatctcctgaaaatcattaaagacaaggacttcctggacaatgaggagaacgaggacattcttgaggacattgtcctcacccttacgttgtttgaagatagggagatgattgaagaacgcttgaaaacttacgctcatctcttcgacgacaaagtcatgaaacagctcaagaggcgccgatatacaggatgggggcggctgtcaagaaaactgatcaatgggatccgagacaagcagagtggaaagacaatcctggattttcttaagtccgatggatttgccaaccggaacttcatgcagttgatccatgatgactctctcacctttaaggaggacatccagaaagcacaagtttctggccagggggacagtcttcacgagcacatcgctaatcttgcaggtagcccagctatcaaaaagggaatactgcagaccgttaaggtcgtggatgaactcgtcaaagtaatgggaaggcataagcccgagaatatcgttatcgagatggcccgagagaaccaaactacccagaagggacagaagaacagtagggaaaggatgaagaggattgaagagggtataaaagaactggggtcccaaatccttaaggaacacccagttgaaaacacccagcttcagaatgagaagctctacctgtactacctgcagaacggcagggacatgtacgtggatcaggaactggacatcaatcggctctccgactacgacgtggctgctatcgtgccccagtcttttctcaaagatgattctattgataataaagtgttgacaagatccgataaagctagagggaagagtgataacgtcccctcagaagaagttgtcaagaaaatgaaaaattattggcggcagctgctgaacgccaaactgatcacacaacggaagttcgataatctgactaaggctgaacgaggtggcctgtctgagttggataaagccggcttcatcaaaaggcagcttgttgagacacgccagatcaccaagcacgtggcccaaattctcgattcacgcatgaacaccaagtacgatgaaaatgacaaactgattcgagaggtgaaagttattactctgaagtctaagctggtctcagatttcagaaaggactttcagttttataaggtgagagagatcaacaattaccaccatgcgcatgatgcctacctgaatgcagtggtaggcactgcacttatcaaaaaatatcccaagcttgaatctgaatttgtttacggagactataaagtgtacgatgttaggaaaatgatcgcaaagtctgagcaggaaataggcaaggccaccgctaagtacttcttttacagcaatattatgaattttttcaagaccgagattacactggccaatggagagattcggaagcgaccacttatcgaaacaaacggagaaacaggagaaatcgtgtgggacaagggtagggatttcgcgacagtccggaaggtcctgtccatgccgcaggtgaacatcgttaaaaagaccgaagtacagaccggaggcttctccaaggaaagtatcctcccgaaaaggaacagcgacaagctgatcgcacgcaaaaaagattgggaccccaagaaatacggcggattcgattctcctacagtcgcttacagtgtactggttgtggccaaagtggagaaagggaagtctaaaaaactcaaaagcgtcaaggaactgctgggcatcacaatcatggagcgatcaagcttcgaaaaaaaccccatcgactttctcgaggcgaaaggatataaagaggtcaaaaaagacctcatcattaagcttcccaagtactctctctttgagcttgaaaacggccggaaacgaatgctcgctagtgcgggcgagctgcagaaaggtaacgagctggcactgccctctaaatacgttaatttcttgtatctggccagccactatgaaaagctcaaagggtctcccgaagataatgagcagaagcagctgttcgtggaacaacacaaacactaccttgatgagatcatcgagcaaataagcgaattctccaaaagagtgatcctcgccgacgctaacctcgataaggtgctttctgcttacaataagcacagggataagcccatcagggagcaggcagaaaacattatccacttgtttactctgaccaacttgggcgcgcctgcagccttcaagtacttcgacaccaccatagacagaaagcggtacacctctacaaaggaggtcctggacgccacactgattcatcagtcaattacggggctctatgaaacaagaatcgacctctctcagctcggtggagacagcagggctgaccccaagaagaagaggaaggtggaggccagcggttccggacgggctgacgcattggacgattttgatctggatatgctgggaagtgacgccctcgatgattttgaccttgacatgcttggttcggatgcccttgatgactttgacctcgacatgctcggcagtgacgcccttgatgatttcgacctggacatgctgattaactctagagcggccgcagatccaaaaaagaagagaaaggtagatccaaaaaagaagagaaaggtagatccaaaaaagaagagaaaggtagatacggccgcatag

SEQ ID NO: 5 - DNA, 587 bp, Artificial
  MS2-activator construct
ccaccatgggacctaagaaaaagaggaaggtggcggccgcttctagaatggcttctaactttactcagttcgttctcgtcgacaatggcggaactggcgacgtgactgtcgccccaagcaacttcgctaacgggatcgctgaatggatcagctctaactcgcgttcacaggcttacaaagtaacctgtagcgttcgtcagagctctgcgcagaatcgcaaatacaccatcaaagtcgaggtgcctaaaggcgcctggcgttcgtacttaaatatggaactaaccattccaattttcgccacgaattccgactgcgagcttattgttaaggcaatgcaaggtctcctaaaagatggaaacccgattccctcagcaatcgcagcaaactccggcatctacgaggccagcggttccggacgggctgacgcattggacgattttgatctggatatgctgggaagtgacgccctcgatgattttgaccttgacatgcttggttcggatgcccttgatgactttgacctcgacatgctcggcagtgacgcccttgatgatttcgacctggacatgctgattaactctagatga

SEQ ID NO: 6 - DNA, 681 bp, Artificial
  MS2-activator construct
gccaccatgggacctaagaaaaagaggaaggtggcggccgcttctagaatggcttctaactttactcagttcgttctcgtcgacaatggcggaactggcgacgtgactgtcgccccaagcaacttcgctaacgggatcgctgaatggatcagctctaactcgcgttcacaggcttacaaagtaacctgtagcgttcgtcagagctctgcgcagaatcgcaaatacaccatcaaagtcgaggtgcctaaaggcgcctggcgttcgtacttaaatatggaactaaccattccaattttcgccacgaattccgactgcgagcttattgttaaggcaatgcaaggtctcctaaaagatggaaacccgattccctcagcaatcgcagcaaactccggcatctacgaggccagcggttccggacgggctgacgcattggacgattttgatctggatatgctgggaagtgacgccctcgatgattttgaccttgacatgcttggttcggatgcccttgatgactttgacctcgacatgctcggcagtgacgcccttgatgatttcgacctggacatgctgattaactctagagcggccgcagatccaaaaaagaagagaaaggtagatccaaaaaagaagagaaaggtagatccaaaaaagaagagaaaggtagatacggccgcatag

SEQ ID NO: 7 - DNA, 557 bp, Artificial
  MS2-activator construct
  misc_feature (320)..(339): wherein N is G, A, T or C
tgtacaaaaaagcaggctttaaaggaaccaattcagtcgactggatccggtaccaaggtcgggcaggaagagggcctatttcccatgattccttcatatttgcatatacgatacaaggctgttagagagataattagaattaatttgactgtaaacacaaagatattagtacaaaatacgtgacgtagaaagtaataatttcttgggtagtttgcagttttaaaattatgttttaaaatggactatcatatgcttaccgtaacttgaaagtatttcgatttcttggctttatatatcttgtggaaaggacgaaacaccgnnnnnnnnnnnnnnnnnnnngttttagagctagaaatagcaagttaaaataaggctagtccgttatcaacttgaaaaagtggcaccgagtcggtgctctgcaggtcgactctagaaaacatgaggatcacccatgtctgcagtattcccgggttcattagatcctaaggtacctaattgcctagaaaacatgaggatcacccatgtctgcaggtcgactctagaaattttttctagac

SEQ ID NO: 8 - DNA, 882 bp, Artificial
  Activation reporter construct
tagggataacagggtaatagtgtcccctccaccccacagtggggcgaggtaggcgtgtacggtgggaggcctatataagcagagctcgtttagtgaaccgtcagatcgcctggagaattcgccaccatggactacaaggatgacgacgataaaacttccggtggcggactgggttccaccgtgagcaagggcgaggaggtcatcaaagagttcatgcgcttcaaggtgcgcatggagggctccatgaacggccacgagttcgagatcgagggcgagggcgagggccgcccctacgagggcacccagaccgccaagctgaaggtgaccaagggcggccccctgcccttcgcctgggacatcctgtccccccagttcatgtacggctccaaggcgtacgtgaagcaccccgccgacatccccgattacaagaagctgtccttccccgagggcttcaagtgggagcgcgtgatgaacttcgaggacggcggtctggtgaccgtgacccaggactcctccctgcaggacggcacgctgatctacaaggtgaagatgcgcggcaccaacttcccccccgacggccccgtaatgcagaagaagaccatgggctgggaggcctccaccgagcgcctgtacccccgcgacggcgtgctgaagggcgagatccaccaggccctgaagctgaaggacggcggccactacctggtggagttcaagaccatctacatggccaagaagcccgtgcaactgcccggctactactacgtggacaccaagctggacatcacctcccacaacgaggactacaccatcgtggaacagtacgagcgctccgagggccgccaccacctgttcctgtacggcatggacgagctgtacaagtaa

SEQ ID NO: 9 - DNA, 882 bp, Artificial
  Activation reporter construct
tagggataacagggtaatagtggggccactagggacaggattggcgaggtaggcgtgtacggtgggaggcctatataagcagagctcgtttagtgaaccgtcagatcgcctggagaattcgccaccatggactacaaggatgacgacgataaaacttccggtggcggactgggttccaccgtgagcaagggcgaggaggtcatcaaagagttcatgcgcttcaaggtgcgcatggagggctccatgaacggccacgagttcgagatcgagggcgagggcgagggccgcccctacgagggcacccagaccgccaagctgaaggtgaccaagggcggccccctgcccttcgcctgggacatcctgtccccccagttcatgtacggctccaaggcgtacgtgaagcaccccgccgacatccccgattacaagaagctgtccttccccgagggcttcaagtgggagcgcgtgatgaacttcgaggacggcggtctggtgaccgtgacccaggactcctccctgcaggacggcacgctgatctacaaggtgaagatgcgcggcaccaacttcccccccgacggccccgtaatgcagaagaagaccatgggctgggaggcctccaccgagcgcctgtacccccgcgacggcgtgctgaagggcgagatccaccaggccctgaagctgaaggacggcggccactacctggtggagttcaagaccatctacatggccaagaagcccgtgcaactgcccggctactactacgtggacaccaagctggacatcacctcccacaacgaggactacaccatcgtggaacagtacgagcgctccgagggccgccaccacctgttcctgtacggcatggacgagctgtacaagtaa

SEQ ID NO: 10 - DNA, 912 bp, Artificial
  Specificity reporter library
  misc_feature (22)..(44): wherein N is G, A, T or C
  misc_feature (154)..(177): wherein N is G, A, T or C
tagggataacagggtaatagtnnnnnnnnnnnnnnnnnnnnnnncgaggtaggcgtgtacggtgggaggcctatataagcagagctcgtttagtgaaccgtcagatcgcctggagaattcgccaccatggactacaaggatgacgacgataaannnnnnnnnnnnnnnnnnnnnnnnacttccggtggcggactgggttccaccgtgagcaagggcgaggaggtcatcaaagagttcatgcgcttcaaggtgcgcatggagggctccatgaacggccacgagttcgagatcgagggcgagggcgagggccgcccctacgagggcacccagaccgccaagctgaaggtgaccaagggcggccccctgcccttcgcctgggacatcctgtccccccagttcatgtacggctccaaggcgtacgtgaagcaccccgccgacatccccgattacaagaagctgtccttccccgagggcttcaagtgggagcgcgtgatgaacttcgaggacggcggtctggtgaccgtgacccaggactcctccctgcaggacggcacgctgatctacaaggtgaagatgcgcggcaccaacttcccccccgacggccccgtaatgcagaagaagaccatgggctgggaggcctccaccgagcgcctgtacccccgcgacggcgtgctgaagggcgagatccaccaggccctgaagctgaaggacggcggccactacctggtggagttcaagaccatctacatggccaagaagcccgtgcaactgcccggctactactacgtggacaccaagctggacatcacctcccacaacgaggactacaccatcgtggaacagtacgagcgctccgagggccgccaccacctgttcctgtacggcatggacgagctgtacaagtaagaattc

SEQ ID NO: 11 - DNA, 23 bp, Artificial
  Target probe
ctggcggatcactcgcggttagg

SEQ ID NO: 12 - DNA, 23 bp, Artificial
  Target probe
cctcggcctccaaaagtgctagg

SEQ ID NO: 13 - DNA, 23 bp, Artificial
  Target probe
acgctgattcctgcagatcaggg

SEQ ID NO: 14 - DNA, 23 bp, Artificial
  Target probe
ccaggaatacgtatccaccaggg

SEQ ID NO: 15 - DNA, 23 bp, Artificial
  Target probe
gccacacccaagcgatcaaatgg

SEQ ID NO: 16 - DNA, 23 bp, Artificial
  Target probe
aaataatacattctaaggtaagg

SEQ ID NO: 17 - DNA, 23 bp, Artificial
  Target probe
gctactggggaggctgaggcagg

SEQ ID NO: 18 - DNA, 23 bp, Artificial
  Target probe
tagcaatacagtcacattaatgg

SEQ ID NO: 19 - DNA, 23 bp, Artificial
  Target probe
ctcatgtgatccccccgtctcgg

SEQ ID NO: 20 - DNA, 23 bp, Artificial
  Target probe
ccgggcagagagtgaacgcgcgg

SEQ ID NO: 21 - DNA, 23 bp, Artificial
  Target probe
ttccttccctctcccgtgcttgg

SEQ ID NO: 22 - DNA, 23 bp, Artificial
  Target probe
tctctgcaaagcccctggagagg

SEQ ID NO: 23 - DNA, 23 bp, Artificial
  Target probe
aatgcagttgccgagtgcagtgg

SEQ ID NO: 24 - DNA, 23 bp, Artificial
  Target probe
cctcagcctcctaaagtgctggg

SEQ ID NO: 25 - DNA, 23 bp, Artificial
  Target probe
gagtccaaatcctctttactagg

SEQ ID NO: 26 - DNA, 23 bp, Artificial
  Target probe
gagtgtctggatttgggataagg

SEQ ID NO: 27 - DNA, 23 bp, Artificial
  Target probe
cagcacctcatctcccagtgagg

SEQ ID NO: 28 - DNA, 23 bp, Artificial
  Target probe
tctaaaacccagggaatcatggg

SEQ ID NO: 29 - DNA, 23 bp, Artificial
  Target probe
cacaaggcagccagggatccagg

SEQ ID NO: 30 - DNA, 23 bp, Artificial
  Target probe
gatggcaagctgagaaacactgg

SEQ ID NO: 31 - DNA, 23 bp, Artificial
  Target probe
tgaaatgcacgcatacaattagg

SEQ ID NO: 32 - DNA, 23 bp, Artificial
  Target probe
ccagtccagacctggccttctgg

SEQ ID NO: 33 - DNA, 23 bp, Artificial
  Target probe
cccagaaaaacagaccctgaagg

SEQ ID NO: 34 - DNA, 23 bp, Artificial
  Target probe
aagggttgagcacttgtttaggg

SEQ ID NO: 35 - DNA, 23 bp, Artificial
  Target probe
atgtctgagttttggttgagagg

SEQ ID NO: 36 - DNA, 23 bp, Artificial
  Target probe
ggtcccttgaaggggaagtaggg

SEQ ID NO: 37 - DNA, 23 bp, Artificial
  Target probe
tggcagtctactcttgaagatgg

SEQ ID NO: 38 - DNA, 23 bp, Artificial
  Target probe
ggcacagtgccagaggtctgtgg

SEQ ID NO: 39 - DNA, 23 bp, Artificial
  Target probe
taaaaataaaaaaactaacaggg

SEQ ID NO: 40 - DNA, 23 bp, Artificial
  Target probe
tctgtgggggacctgcactgagg

SEQ ID NO: 41 - DNA, 23 bp, Artificial
  Target probe
ggccagaggtcaaggctagtggg

SEQ ID NO: 42 - DNA, 23 bp, Artificial
  Target probe
cacgaccgaaacccttcttacgg

SEQ ID NO: 43 - DNA, 23 bp, Artificial
  Target probe
gttgaatgaagacagtctagtgg

SEQ ID NO: 44 - DNA, 23 bp, Artificial
  Target probe
taagaacagagcaagttacgtgg

SEQ ID NO: 45 - DNA, 23 bp, Artificial
  Target probe
tgtaaggtaagagaggagagcgg

SEQ ID NO: 46 - DNA, 23 bp, Artificial
  Target probe
tgacacaccaactcctgcactgg

SEQ ID NO: 47 - DNA, 23 bp, Artificial
  Target probe
tttacccacttccttcgaaaagg

SEQ ID NO: 48 - DNA, 23 bp, Artificial
  Target probe
gtggctggcaggctggctctggg

SEQ ID NO: 49 - DNA, 23 bp, Artificial
  Target probe
ctcccccggcctcccccgcgcgg

SEQ ID NO: 50 - DNA, 23 bp, Artificial
  Target probe
caaaacccggcagcgaggctggg

SEQ ID NO: 51 - DNA, 23 bp, Artificial
  Target probe
aggagccgccgcgcgctgattgg

SEQ ID NO: 52 - DNA, 23 bp, Artificial
  Target probe
cacacacacccacacgagatggg

SEQ ID NO: 53 - DNA, 23 bp, Artificial
  Target probe
gaagaagctaaagagccagaggg

SEQ ID NO: 54 - DNA, 23 bp, Artificial
  Target probe
atgagaatttcaataacctcagg

SEQ ID NO: 55 - DNA, 23 bp, Artificial
  Target probe
tcccgctctgttgcccaggctgg

SEQ ID NO: 56 - DNA, 23 bp, Artificial
  Target probe
cagacacccaccaccatgcgtgg

SEQ ID NO: 57 - DNA, 23 bp, Artificial
  Target probe
tcccaatttactgggattacagg

SEQ ID NO: 58 - DNA, 23 bp, Artificial
  Target probe
tgatttaaaagttggaaacgtgg

SEQ ID NO: 59 - DNA, 23 bp, Artificial
  Target probe
tctagttccccacctagtctggg

SEQ ID NO: 60 - DNA, 23 bp, Artificial
  Target probe
gattaactgagaattcacaaggg

SEQ ID NO: 61 - DNA, 23 bp, Artificial
  Target probe
cgccaggaggggtgggtctaagg

SEQ ID NO: 62 - DNA, 23 bp, Artificial
  Reporter construct
gtcccctccaccccacagtgggg

SEQ ID NO: 63 - DNA, 23 bp, Artificial
  Reporter construct
ggggccactagggacaggattgg

SEQ ID NO: 64 - DNA, 71 bp, Artificial
  Target oligonucleotide sequence
taatacttttatctgtcccctccaccccacagtggggccactagggacaggattggtgacagaaaagcccc

SEQ ID NO: 65 - DNA, 20 bp, Artificial
  Target oligonucleotide sequence
ggggccactagggacaggat

SEQ ID NO: 66 - RNA, 80 nt, Artificial
  Guide RNA
guuuuagagcuagaaauagcaaguuaaaauaaggcuagcuuguuaucaacuugaaaaaguggcaccgagucggugcuuuu

SEQ ID NO: 67 - DNA, 23 bp, Artificial
  Target oligonucleotide sequence
gtcccctccaccccacagtgcag

SEQ ID NO: 68 - DNA, 23 bp, Artificial
  Target oligonucleotide sequence
gtcccctccaccccacagtgcaa

SEQ ID NO: 69 - DNA, 23 bp, Artificial
  Target oligonucleotide sequence
gtcccctccaccccacagtgcgg

SEQ ID NO: 70 - DNA, 52 bp, Artificial
  Target oligonucleotide sequence
tgtcccctccaccccacagtggggccactagggacaggattggtgacagaaa

SEQ ID NO: 71 - DNA, 52 bp, Artificial
  Target oligonucleotide sequence
tgtcccccccaccccacagtggggccactagggacaggattggtgacagaaa

SEQ ID NO: 72 - DNA, 52 bp, Artificial
  Target oligonucleotide sequence
aaaaccctccaccccacagtggggccactagggacaggattggtgacagaaa

SEQ ID NO: 73 - DNA, 52 bp, Artificial
  Target oligonucleotide sequence
tgtcccctccttttttcagtggggccactagggacaggattggtgacagaaa

SEQ ID NO: 74 - DNA, 23 bp, Artificial
  Target oligonucleotide sequence
caccggggtggtgcccatcctgg

SEQ ID NO: 75 - DNA, 23 bp, Artificial
  Target oligonucleotide sequence
ggtgcccatcctggtcgagctgg

SEQ ID NO: 76 - DNA, 23 bp, Artificial
  Target oligonucleotide sequence
cccatcctggtcgagctggacgg

SEQ ID NO: 77 - DNA, 23 bp, Artificial
  Target oligonucleotide sequence
ggccacaagttcagcgtgtccgg

SEQ ID NO: 78 - DNA, 23 bp, Artificial
  Target oligonucleotide sequence
cgcaaataagagctcacctacgg

SEQ ID NO: 79 - DNA, 23 bp, Artificial
  Target oligonucleotide sequence
ctgaagttcatctgcaccaccgg

SEQ ID NO: 80 - DNA, 23 bp, Artificial
  Target oligonucleotide sequence
ccggcaagctgcccgtgccctgg

SEQ ID NO: 81 - DNA, 23 bp, Artificial
  Target oligonucleotide sequence
gaccaggatgggcaccaccccgg

SEQ ID NO: 82 - DNA, 23 bp, Artificial
  Target oligonucleotide sequence
gccgtccagctcgaccaggatgg

SEQ ID NO: 83 - DNA, 23 bp, Artificial
  Target oligonucleotide sequence
ggccggacacgctgaacttgtgg

SEQ ID NO: 84 - DNA, 23 bp, Artificial
  Target oligonucleotide sequence
taacagggtaatgtcgaggccgg

SEQ ID NO: 85 - DNA, 23 bp, Artificial
  Target oligonucleotide sequence
aggtgagctcttatttgcgtagg

SEQ ID NO: 86 - DNA, 23 bp, Artificial
  Target oligonucleotide sequence
cttcagggtcagcttgccgtagg

SEQ ID NO: 87 - DNA, 23 bp, Artificial
  Target oligonucleotide sequence
gggcacgggcagcttgccggtgg

SEQ ID NO: 88 - DNA, 23 bp, Artificial
  Target oligonucleotide sequence
gagatgatcgccccttcttctgg

SEQ ID NO: 89 - DNA, 20 bp, Artificial
  Target oligonucleotide sequence
gagatgatcgccccttcttc

SEQ ID NO: 90 - DNA, 20 bp, Artificial
  Target oligonucleotide sequence
gtgatgaccggccgttcttc

SEQ ID NO: 91 - DNA, 23 bp, Artificial
  Target oligonucleotide sequence
gtcccctccaccccacagtgggg

SEQ ID NO: 92 - DNA, 23 bp, Artificial
  Target oligonucleotide sequence
gagatgatcgcccgttcttctgg

SEQ ID NO: 93 - RNA, 20 nt, Artificial
  RNA target sequence
guccccuccaccccacagug

SEQ ID NO: 94 - RNA, 20 nt, Artificial
  RNA target sequence
guccccuccaccccacaguc

SEQ ID NO: 95 - RNA, 20 nt, Artificial
  RNA target sequence
guccccuccaccccacagag

SEQ ID NO: 96 - RNA, 20 nt, Artificial
  RNA target sequence
guccccuccaccccacacug

SEQ ID NO: 97 - RNA, 20 nt, Artificial
  RNA target sequence
guccccuccaccccacugug

SEQ ID NO: 98 - RNA, 20 nt, Artificial
  RNA target sequence
guccccuccaccccagagug

SEQ ID NO: 99 - RNA, 20 nt, Artificial
  RNA target sequence
guccccuccaccccucagug

SEQ ID NO: 100 - RNA, 20 nt, Artificial
  RNA target sequence
guccccuccacccgacagug

SEQ ID NO: 101 - RNA, 20 nt, Artificial
  RNA target sequence
guccccuccaccgcacagug

SEQ ID NO: 102 - RNA, 20 nt, Artificial
  RNA target sequence
guccccuccacgccacagug

SEQ ID NO: 103 - RNA, 20 nt, Artificial
  RNA target sequence
guccccuccagcccacagug

SEQ ID NO: 104 - RNA, 20 nt, Artificial
  RNA target sequence
guccccuccuccccacagug

SEQ ID NO: 105 - RNA, 20 nt, Artificial
  RNA target sequence
guccccucgaccccacagug

SEQ ID NO: 106 - RNA, 20 nt, Artificial
  RNA target sequence
guccccuccaccccacagac

SEQ ID NO: 107 - RNA, 20 nt, Artificial
  RNA target sequence
guccccuccaccccacucug

SEQ ID NO: 108 - RNA, 20 nt, Artificial
  RNA target sequence
guccccuccaccccugagug

SEQ ID NO: 109 - RNA, 20 nt, Artificial
  RNA target sequence
guccccuccaccggacagug

SEQ ID NO: 110 - RNA, 20 nt, Artificial
  RNA target sequence
guccccuccaggccacagug

SEQ ID NO: 111 - RNA, 20 nt, Artificial
  RNA target sequence
guccccucguccccacagug

SEQ ID NO: 112 - DNA, 23 bp, Artificial
  Target oligonucleotide sequence
ggggccactagggacaggatggg

SEQ ID NO: 113 - RNA, 20 nt, Artificial
  RNA target sequence
gagaugaucgccccuucuuc

SEQ ID NO: 114 - RNA, 20 nt, Artificial
  RNA target sequence
gagaugaucgccccuucuug

SEQ ID NO: 115 - RNA, 20 nt, Artificial
  RNA target sequence
gagaugaucgccccuucuac

SEQ ID NO: 116 - RNA, 20 nt, Artificial
  RNA target sequence
gagaugaucgccccuucauc

SEQ ID NO: 117 - RNA, 20 nt, Artificial
  RNA target sequence
gagaugaucgccccuuguuc

SEQ ID NO: 118 - RNA, 20 nt, Artificial
  RNA target sequence
gagaugaucgccccuacuuc

SEQ ID NO: 119 - RNA, 20 nt, Artificial
  RNA target sequence
gagaugaucgccccaucuuc

SEQ ID NO: 120 - RNA, 20 nt, Artificial
  RNA target sequence
gagaugaucgcccguucuuc

SEQ ID NO: 121 - RNA, 20 nt, Artificial
  RNA target sequence
gagaugaucgccgcuucuuc

SEQ ID NO: 122 - RNA, 20 nt, Artificial
  RNA target sequence
gagaugaucgcgccuucuuc

SEQ ID NO: 123 - RNA, 20 nt, Artificial
  RNA target sequence
gagaugaucggcccuucuuc

SEQ ID NO: 124 - RNA, 20 nt, Artificial
  RNA target sequence
gagaugauccccccuucuuc

SEQ ID NO: 125 - RNA, 20 nt, Artificial
  RNA target sequence
gagaugauggccccuucuuc

SEQ ID NO: 126 - RNA, 20 nt, Artificial
  RNA target sequence
gagaugaucgccccuucuag

SEQ ID NO: 127 - RNA, 20 nt, Artificial
  RNA target sequence
gagaugaucgccccuugauc

SEQ ID NO: 128 - RNA, 20 nt, Artificial
  RNA target sequence
gagaugaucgccccaacuuc

SEQ ID NO: 129 - RNA, 20 nt, Artificial
  RNA target sequence
gagaugaucgccgguucuuc

SEQ ID NO: 130 - RNA, 20 nt, Artificial
  RNA target sequence
gagaugaucgggccuucuuc

SEQ ID NO: 131 - RNA, 20 nt, Artificial
  RNA target sequence
gagaugaugcccccuucuuc

SEQ ID NO: 132 - DNA, 23 bp, Artificial
  Target oligonucleotide sequence
gagatgatcgccccttcttctgg

SEQ ID NO: 133 - RNA, 20 nt, Artificial
  RNA target sequence
ggggccacuagggacaggau

SEQ ID NO: 134 - RNA, 19 nt, Artificial
  RNA target sequence
gggccacuagggacaggau

SEQ ID NO: 135 - RNA, 18 nt, Artificial
  RNA target sequence
ggccacuagggacaggau

SEQ ID NO: 136 - RNA, 17 nt, Artificial
  RNA target sequence
gccacuagggacaggau

SEQ ID NO: 137 - RNA, 20 nt, Artificial
  RNA target sequence
gagaugaucgccccuucuuc

SEQ ID NO: 138 - RNA, 18 nt, Artificial
  RNA target sequence
gaugaucgccccuucuuc

SEQ ID NO: 139 - RNA, 15 nt, Artificial
  RNA target sequence
gaucgccccuucuuc

SEQ ID NO: 140 - RNA, 11 nt, Artificial
  RNA target sequence
gccccuucuuc

SEQ ID NO: 141 - DNA, 21 bp, Artificial
  Target oligonucleotide sequence
gtcccctccaccccacagtgc

SEQ ID NO: 142 - DNA, 14 bp, Artificial
  Target oligonucleotide sequence
  misc_feature (5)..(10): wherein N id G, A, T or C
tgtcnnnnnnaccc

SEQ ID NO: 143 - DNA, 14 bp, Artificial
  Target oligonucleotide sequence
tgtcaaaaaaaccc

SEQ ID NO: 144 - DNA, 14 bp, Artificial
  Target oligonucleotide sequence
tgtcggggggaccc

SEQ ID NO: 145 - DNA, 14 bp, Artificial
  Target oligonucleotide sequence
tgtcaaaaaaaccc

SEQ ID NO: 146 - DNA, 14 bp, Artificial
  Target oligonucleotide sequence
tgtcggggggaccc

SEQ ID NO: 147 - DNA, 14 bp, Artificial
  Target oligonucleotide sequence
tgtcccccccaccc

SEQ ID NO: 148 - DNA, 14 bp, Artificial
  Target oligonucleotide sequence
tgtcttttttaccc

SEQ ID NO: 149 - DNA, 14 bp, Artificial
  Target oligonucleotide sequence
tgtcccccccaccc

SEQ ID NO: 150 - DNA, 14 bp, Artificial
  Target oligonucleotide sequence
tgtcttttttaccc

SEQ ID NO: 151 - DNA, 23 bp, Artificial
  Target oligonucleotide sequence
ggatcctgtgtccccgagctggg

SEQ ID NO: 152 - DNA, 23 bp, Artificial
  Target oligonucleotide sequence
gttaatgtggctctggttctggg

SEQ ID NO: 153 - DNA, 23 bp, Artificial
  Target oligonucleotide sequence
ggggccactagggacaggattgg

SEQ ID NO: 154 - DNA, 23 bp, Artificial
  Target oligonucleotide sequence
cttcctagtctcctgatattggg

SEQ ID NO: 155 - DNA, 23 bp, Artificial
  Target oligonucleotide sequence
tggtcccagctcggggacacagg

SEQ ID NO: 156 - DNA, 23 bp, Artificial
  Target oligonucleotide sequence
agaaccagagccacattaaccgg

SEQ ID NO: 157 - DNA, 23 bp, Artificial
  Target oligonucleotide sequence
gtcaccaatcctgtccctagtgg

SEQ ID NO: 158 - DNA, 23 bp, Artificial
  Target oligonucleotide sequence
agacccaatatcaggagactagg

SEQ ID NO: 159 - DNA, 75 bp, Artificial
  Target oligonucleotide sequence
gggatcctgtgtccccgagctgggaccaccttatattcccagggccggttaatgtggctctggttctgggtactt

SEQ ID NO: 160 - DNA, 69 bp, Artificial
  Target oligonucleotide sequence
gggatcctgtgtccccgagctgggaccaccttatattcccagggccggttaatgtggttctgggtactt

SEQ ID NO: 161 - DNA, 113 bp, Artificial
  Target oligonucleotide sequence
gggatcctgtgtccccgagctgggaccaccttatattcccagggcagggccggttggaccaccttatattcccagggcagggccggttaatgtggctctggttctgggtactt

SEQ ID NO: 162 - DNA, 34 bp, Artificial
  Target oligonucleotide sequence
gggatcctgtgtccccgtctggttctgggtactt

SEQ ID NO: 163 - DNA, 47 bp, Artificial
  Target oligoncleotide sequence
gggatcctgtgtccccgagctgggaccaccttatattctgggtactt

SEQ ID NO: 164 - DNA, 17 bp, Artificial
  Target oligonucleotide sequence
gggatcctgtggtactt

SEQ ID NO: 165 - DNA, 93 bp, Artificial
  Target oligonucleotide sequence
agggccggttaatgtggctctggttctgggtacttttatctgtcccctccaccccacagtggggccactagggacaggattggtgacagaaaa

SEQ ID NO: 166 - DNA, 83 bp, Artificial
  Target oligonucleotide sequence
agggccggttaatgaatgtggctctggttctgggtacttttatctgtcccctccaccccacagtggggccactagacagaaaa

SEQ ID NO: 167 - DNA, 76 bp, Artificial
  Target oligonucleotide sequence
agggccggttaatgtggctctggttctgggtacttttatctgtcccccagtggggccactgattggtgacagaaaa

SEQ ID NO: 168 - DNA, 29 bp, Artificial
  Target oligonucleotide sequence
agggccggttcaggattggtgacagaaaa

SEQ ID NO: 169 - DNA, 34 bp, Artificial
  Target oligonucleotide sequence
agggccggttaatgtggcgattggtgacagaaaa

SEQ ID NO: 170 - DNA, 63 bp, Artificial
  Target oligonucleotide sequence
agggccggttaatgtggctctggttctgggtacttttatctgtccccgattggtgacagaaaa

SEQ ID NO: 171 - DNA, 84 bp, Artificial
  Target oligonucleotide sequence
agggccggttaatgtggctctggttctgggtacttttatctgtcccctccaccccacagtggggacaggattggtgacagaaaa

SEQ ID NO: 172 - DNA, 27 bp, Artificial
  Target oligonucleotide sequence
agggccggttaatgtggtgacagaaaa

SEQ ID NO: 173 - DNA, 105 bp, Artificial
  Target oligonucleotide sequence
agggccggttaatgtggctctggttctgggtacttttatctgtcccctccaccccaggggacagtctgtcccctccaccccagggacaggattggtgacagaaaa

SEQ ID NO: 174 - DNA, 80 bp, Artificial
  Target oligonucleotide sequence
agggccggttaatgtggctctggttctgggtacttttatctgtcccctccaccactagggacaggattggtgacagaaaa

SEQ ID NO: 175 - DNA, 53 bp, Artificial
  Target oligonucleotide sequence
cccacagtggggccactagggacaggattggtgacagaaaagccccatacccc

SEQ ID NO: 176 - DNA, 22 bp, Artificial
  Target oligonucleotide sequence
cccacagtggggccactacccc

SEQ ID NO: 177 - DNA, 96 bp, Artificial
  Target oligonucleotide sequence
cccacagtggggccactagtagaaaagccccatccttaggcctcccccatccttaggcctcctccttcctagtctcctgatattgggtctaacccc

SEQ ID NO: 178 - DNA, 94 bp, Artificial
  Target oligonucleotide sequence
cccacagtggggccactagggacaggattggtgacagaaaagccccatccttaggcctcctccttcctagtctcctgatattgggtctaacccc

SEQ ID NO: 179 - DNA, 62 bp, Artificial
  Target oligonucleotide sequence
cccacagtggggccacccttaggcctcctccttcctagtctcctgatattgggtctaacccc

SEQ ID NO: 180 - DNA, 38 bp, Artificial
  Target oligonucleotide sequence
cccacagtggggccactagtgatattgggtctaacccc

SEQ ID NO: 181 - DNA, 94 bp, Artificial
  target oligonucleotide sequence
cccacagtggggccactagggacaggattggtgacaaaaaagccccatccttacgcctcctccttcctagtctcctgatattgggtctaacccc

SEQ ID NO: 182 - DNA, 65 bp, Artificial
  Target oligonucleotide sequence
cccacagtggggccactagggacaggcctcctccttcctagtctcctgatattgggtctaacccc

SEQ ID NO: 183 - DNA, 102 bp, Artificial
  Target oligonucleotide sequence
cccacagtggggccactagggacagggggacaggattggtgacagaaaagccccatccttaggcctcctccttcctagtctcctgatattgggtctaacccc

SEQ ID NO: 184 - DNA, 76 bp, Artificial
  Target oligonucleotide sequence
cccacaggattggtgacagaaaagccccatccttaggcctcctccttcctagtctcctgatattgggtctaacccc